European Patent Application EP 4 183 883 A1, published May 24, 2023. Title: THRAUSTOCHYTRIDS, FATTY ACID COMPOSITIONS, AND METHODS OF MAKING AND USES THEREOF. Applicant: DSM IP Assets B.V. The sequence listing filed with the application follows.

SEQUENCE LISTING (5 sequences)

SEQ ID NO: 1 - DNA, 1713 bp, Schizochytrium sp.
  source 1..1713: mol_type = unassigned DNA
acctggttgatcctgccagctgtcatttgctcgtctaaaagattaagccatgcatgtctaagtataaacaaattatacggtgaaactgcgaacggctcattatatcagttatagtttctttgatagtgtatttctatatctatttggataactgtggcaattctagagctaacacatgctttcgagtgggactttttggtaccactgcatttattagattttgaagccaacgtaaaattggtgattcatgataactttgcgaatcgcagtagcgtcttgtacgcggcgatgaatcattcaagtttctgccccatcagctgtcgatggtacggtattggcctaccatggctttcacgggtgacggagaattagggtttgattccggagaggacgcttgagagacggcgaccacatccaaggaaggcagcaggcgcgtaaattacccaatggggactccccgaggtagtgacaagaaataaaaatgaggagcgctttgcgtttttcaatttgaatgagagaatcgtacaatcctcatcgaggatcaattggagggcaagtctggtgccagcagccgcggtaactccagctccaatagcaaatattagagttgttgcagttaaaaagctcgtagttgaatttccgatagtctttggccgtgtccttggtctcgtatcatgggtttattgtgccaagatgatcgtcctctatggttagtgatagtcatagtcgtttactgtaaaaaaactggagtgtttaaagcatttctttgggaaaggtacatattagtataggataattagataggacctgtgattcttatttggttggtttgtgagtcatggtaatgattaatagggacaatcgggggtattcgaatttaattgtcagaggtgaaattcttggatttaagaaagtcgaactactgcgaaggcatttaccaaggatgttttcattaataaagaacgaaagttaggggatcgaagatgattagataccatcgtagtcttaactgtaaactatgccgacttgcgattgtccgtcgttgttttttcaaaaaagagacctgggcagcagcacatgagaaatcaaagtttttgggttccggggggagtatggtcgcaaggctgaaacttaaaggaattgacggaagggcaccaccaggagtggagcctgcggcttaattcgactcaacacgggaaaacttaccaggtccagacatagtaaggattgacagattgagagctctttcttgattctatgggtggtggtgcatggccgttcttagttggtggagtgatttgtctggttaattccgttaacgaacgagacctcagcctactaaatagtggtgcatattgtgagatatgtgacaaaaatcgcttcttagagggacatttcgggtttaccggaaggaagtttgaggcaataacaggtctgtgatgcccctagatgttctgggccgcacgcgcgctacaatgacagattcaacaagtccggtagtggagcttttgcttctctattattacttttccgagaggaatggttaatcttctaaatgtctgtcgtgatggggctagatttttgcaattattaatctccaacgaggaattcctagtaaacgcaagtcatcagcttgcattgattacgtccctgccctttgtacacaccgcccgtcgcacctaccgattgaacggtcctatgaaatcttcggat

SEQ ID NO: 2 - DNA, 924 bp, Schizochytrium sp.
  source 1..924: mol_type = unassigned DNA
atcgaccagaaggatgcctacgtaggggacgaggcgcagagcaagcgtggtgtgctgacgctcaagtacccgatcgagcacggcatcgtgaccaactgggacgacatggagaagatctggcatcacaccttctacaacgagctgcgcgtggcgcccgaggagcaccccgtgctgctcaccgaggcccccctcaaccccaaggcgaaccgcgagcgcatgacccagatcatgttcgagaccttcaacgtgccggccatgtacgtcaacatccaggccgtgctgtccctgtacgcttcgggccgcaccaccggcgccgtgctcgattcgggagatggcgtcacgcacaccgtgcccatctacgagggctacgcgctcccgcacgcggtgctgcgcatcgacctggctggccgcgacctgaccgactacatgatgaagatcctgacggagcgcgggtactcgttcacgacgaccgccgagcgcgaaatcgtgcgcgacatcaaggagaagctgtgctacgtggcgctcgacttcgaccaggagatgaagacggccgccgagtcgtcgtcgctggagaagagctacgagctgccggacggcaacgtgatcacgatcggcaacgagcgcttccgctgccccgaggtgctcttccagccgtcgttcatcggcaaggaggccgccggcgtgcacgagaccatgttccagacgatcatgaagtgcgacgtcgatatccgcaaggacctgtacgccaacatcgtcatgtccggtggctccaccatgtacgagggcatcgccgcgcgcctggagaaggagatggtgtcactggcgccctccaccatgaagatcaaggtggtcgcgccccccgagcgcaagtactcggtgtggatcggcggctccatcctggcctcgctctccaccttccagcaa

SEQ ID NO: 3 - protein, 291 aa, Schizochytrium sp.
VLTLKYPIEHGIVTNWDDMEKIWHHTFYNELRVAPEEHPVLLTEAPLNPKANRERMTQIMFETFNVPAMYVNIQAVLSLYASGRTTGAVLDSGDGVTHTVPIYEGYALPHAVLRIDLAGRDLTDYMMKILTERGYSFTTTAEREIVRDIKEKLCYVALDFDQEMKTAAESSSLEKSYELPDGNVITIGNERFRCPEVLFQPSFIGKEAAGVHETMFQTIMKCDVDIRKDLYANIVMSGGSTMYEGIAARLEKEMVSLAPSTMKIKVVAPPERKYSVWIGGSILASLSTFQQ

SEQ ID NO: 4 - DNA, 918 bp, Schizochytrium sp.
  source 1..918: mol_type = unassigned DNA
gatctgcagctggagcgcatcaacgtgtacttcaacgaggccacgggcggccgctacgtgccgcgcgccatcctcatggacctggagcccggtacgatggactctgtccgcgccggcccctttggccagctcttccgcccagacaacttcgtcttcgggcagacgggcgccggtaacaactgggccaagggccactacactgagggcgcggagcttatcgactcggtgctcgacgtggtgcgcaaggaggcagagtcgtgcgactgcctgcagggcttccagatcacccactcgctcggcggcggcacgggctccggtatgggcacgcttctcatcagcaagatccgcgaggagtaccccgaccgcatcatgctgaccttctccatcgtgccctcgcccaaggtgtcggacaccgtcgtggagccctacaacgcgacgctctcggtgcaccagctcgtggagaacgccgacgaggtcatggtcctcgacaacgaggcgctgtacgacatctgcttccgcaccttgaagctcaccacgcccacctacggcgacctcaaccacctcgtgtgcgccgccatgagcgggtgcacgtgctgcctgcgcttcccgggccagctcaactcggacctgcgcaagctggccgtcaacctggtgccctttccgcgcctccacttcttcatgatcggcttctcgcccctcacctcgcgtggctcgcagcagtaccgcgccctgaccgttccggagctcacgcagcaggcgtttgacgctaagaacatgatgtgcgccgccgacccgcgccacggccgctacctgacggcgacgacgctcttccgcgggcgcatgtcgaccaaggaggtggacgagcagatgctcaacatccagaacaagaactcgtcgtactttgtcgagtggatcccc

SEQ ID NO: 5 - protein, 307 aa, Schizochytrium sp.
DDLQLERINVYFNEATGGRYVPRAILMDLEPGTMDSVRAGPFGQLFRPDNFVFGQTGAGNNWAKGHYTEGAELIDSVLDVVRKEAESCDCLQGFQITHSLGGGTGSGMGTLLISKIREEYPDRIMLTFSIVPSPKVSDTVVEPYNATLSVHQLVENADEVMVLDNEALYDICFRTLKLTTPTYGDLNHLVCAAMSGCTCCLRFPGQLNSDLRKLAVNLVPFPRLHFFMIGFSPLTSRGSQQYRALTVPELTQQAFDAKNMMCAADPRHGRYLTATTLFRGRMSTKEVDEQMLNIQNKNSSYFVEWIP